European Patent Specification EP 3 209 306 B1, published April 24, 2024. Title: STABLE NEURAL STEM CELLS COMPRISING AN EXOGENOUS POLYNUCLEOTIDE CODING FOR A GROWTH FACTOR AND METHODS OF USE THEREOF. Applicant: Neuralstem, Inc. The sequence listing filed with the application follows.

SEQUENCE LISTING (3 sequences)

SEQ ID NO: 1 - DNA, 477 bp, Artificial sequence
  Synthesized: IGF-1 isoform 4 cDNA
atgggaaaaatcagcagtcttccaacccaattatttaagtgctgcttttgtgatttcttgaaggtgaagatgcacaccatgtcctcctcgcatctcttctacctggcgctgtgcctgctcaccttcaccagctctgccacggctggaccggagacgctctgcggggctgagctggtggatgctcttcagttcgtgtgtggagacaggggcttttatttcaacaagcccacagggtatggctccagcagtcggagggcgcctcagacaggcatcgtggatgagtgctgcttccggagctgtgatctaaggaggctggagatgtattgcgcacccctcaagcctgccaagtcagctcgctctgtccgtgcccagcgccacaccgacatgcccaagacccagaagtatcagcccccatctaccaacaagaacacgaagtctcagagaaggaaaggaagtacatttgaagaacgcaagtag

SEQ ID NO: 2 - protein, 158 aa, Artificial sequence
  Synthesized: IGF-1 isoform 4 protein
MGKISSLPTQLFKCCFCDFLKVKMHTMSSSHLFYLALCLLTFTSSATAGPETLCGAELVDALQFVCGDRGFYFNKPTGYGSSSRRAPQTGIVDECCFRSCDLRRLEMYCAPLKPAKSARSVRAQRHTDMPKTQKYQPPSTNKNTKSQRRKGSTFEERK

SEQ ID NO: 3 - DNA, 1217 bp, Artificial sequence
  Synthesized: human ubiquitin C promoter
gatctggcctccgcgccgggttttggcgcctcccgcgggcgcccccctcctcacggcgagcgctgccacgtcagacgaagggcgcagcgagcgtcctgatccttccgcccggacgctcaggacagcggcccgctgctcataagactcggccttagaaccccagtatcagcagaaggacattttaggacgggacttgggtgactctagggcactggttttctttccagagagcggaacaggcgaggaaaagtagtcccttctcggcgattctgcggagggatctccgtggggcggtgaacgccgatgattatataaggacgcgccgggtgtggcacagctagttccgtcgcagccgggatttgggtcgcggttcttgtttgtggatcgctgtgatcgtcacttggtgagtagcgggctgctgggctggccggggctttcgtggccgccgggccgctcggtgggacggaagcgtgtggagagaccgccaagggctgtagtctgggtccgcgagcaaggttgccctgaactgggggttggggggagcgcagcaaaatggcggctgttcccgagtcttgaatggaagacgcttgtgaggcgggctgtgaggtcgttgaaacaaggtggggggcatggtgggcggcaagaacccaaggtcttgaggccttcgctaatgcgggaaagctcttattcgggtgagatgggctggggcaccatctggggaccctgacgtgaagtttgtcactgactggagaactcgggtttgtcgtctggttgcgggggcggcagttatgcggtgccgttgggcagtgcacccgtacctttgggagcgcgcgcctcgtcgtgtcgtgacgtcacccgttctgttggcttataatgcagggtggggccacctgccggtaggtgtgcggtaggcttttctccgtcgcaggacgcagggttcgggcctagggtaggctctcctgaatcgacaggcgccggacctctggtgaggggagggataagtgaggcgtcagtttctttggtcggttttatgtacctatcttcttaagtagctgaagctccggttttgaactatgcgctcggggttggcgagtgtgttttgtgaagttttttaggcaccttttgaaatgtaatcatttgggtcaatatgtaattttcagtgttagactagtaaattgtccgctaaattctggccgtttttggcttttttgttagac